European Patent Specification EP 3 749 781 B1, published October 2, 2024. Title: FAR-RED DYE PROBE FORMULATIONS. Applicant: GEN-PROBE INCORPORATED AUBIN-WALKER, Sheila MAJLESSI, Mehrdad R. BOUSQUET, Joshua PHAM, Jimmykim. Application TBA. The sequence listing filed with the application follows.

SEQUENCE LISTING (20 sequences)

SEQ ID NO: 1 - DNA, 45 bp, Artificial Sequence
  Synthetic Oligonucleotide
  misc_feature (13)..(45)
ucuguuaguucctttaaaaaaaaaaaaaaaaaaaaaaaaaaaaaa

SEQ ID NO: 2 - DNA, 16 bp, Artificial Sequence
  Synthetic Oligonucleotide
cggatgggtgagtaac

SEQ ID NO: 3 - DNA, 45 bp, Artificial Sequence
  Synthetic Oligonucleotide
  promoter (1)..(27)
aatttaatacgactcactatagggagataagcccttaccttacca

SEQ ID NO: 4 - DNA, 45 bp, Artificial Sequence
  Synthetic Oligonucleotide
  promoter (1)..(27)
aatttaatacgactcactatagggagataagccgttaccttacca

SEQ ID NO: 5 - DNA, 26 bp, Artificial Sequence
  Synthetic Oligonucleotide
gucugggauaccacuuggaaacagac

SEQ ID NO: 6 - DNA, 21 bp, Artificial Sequence
  Synthetic Oligonucleotide
cacucacgcaugucuagagug

SEQ ID NO: 7 - DNA, 50 bp, Artificial Sequence
  Synthetic Oligonucleotide
  misc_feature (18)..(50)
caugcuccgccgcuugutttaaaaaaaaaaaaaaaaaaaaaaaaaaaaaa

SEQ ID NO: 8 - DNA, 25 bp, Artificial Sequence
  Synthetic Oligonucleotide
cttacctgggcttgacatgtgcctg

SEQ ID NO: 9 - DNA, 45 bp, Artificial Sequence
  Synthetic Oligonucleotide
  promoter (1)..(27)
aatttaatacgactcactatagggagacaccacctgtgaacctgc

SEQ ID NO: 10 - DNA, 24 bp, Artificial Sequence
  Synthetic Oligonucleotide
ccugcagagaugugguuucgcagg

SEQ ID NO: 11 - DNA, 54 bp, Artificial Sequence
  Synthetic Oligonucleotide
  misc_feature (22)..(54)
guaccgucgaugucuucccugtttaaaaaaaaaaaaaaaaaaaaaaaaaaaaaa

SEQ ID NO: 12 - DNA, 16 bp, Artificial Sequence
  Synthetic Oligonucleotide
agcgttatccggattc

SEQ ID NO: 13 - DNA, 51 bp, Artificial Sequence
  Synthetic Oligonucleotide
  promoter (1)..(27)
aatttaatacgactcactatagggagattcggaacccggctcgagcttaag

SEQ ID NO: 14 - DNA, 24 bp, Artificial Sequence
  Synthetic Oligonucleotide
ccgcucaggcgguugcucaagcgg

SEQ ID NO: 15 - DNA, 24 bp, Artificial Sequence
  Synthetic Oligonucleotide
ccgcucaggcgguugcucaagcgg

SEQ ID NO: 16 - DNA, 57 bp, Artificial Sequence
  Synthetic Oligonucleotide
  misc_feature (25)..(57)
cguucacuauuggucucugcauuctttaaaaaaaaaaaaaaaaaaaaaaaaaaaaaa

SEQ ID NO: 17 - DNA, 19 bp, Artificial Sequence
  Synthetic Oligonucleotide
gattatataggacgacaag

SEQ ID NO: 18 - DNA, 49 bp, Artificial Sequence
  Synthetic Oligonucleotide
  promoter (1)..(27)
aatttaatacgactcactatagggagagatgattgacttgtgattccgc

SEQ ID NO: 19 - DNA, 23 bp, Artificial Sequence
  Synthetic Oligonucleotide
gcauggugcgaauugggacaugc

SEQ ID NO: 20 - DNA, 14 bp, Artificial Sequence
  Synthetic Oligonucleotide
tttttttttttttt